European Patent Specification EP 3 518 961 B1, published February 22, 2023. Title: PTH compounds with low peak-to-trough ratios. Applicant: Ascendis Pharma A/S. The sequence listing filed with the application follows.

SEQUENCE LISTING (122 sequences)

SEQ ID NO: 1 - protein, 84 aa, Homo sapiens
SVSEIQLMHNLGKHLNSMERVEWLRKKLQDVHNFVALGAPLAPRDAGSQRPRKKEDNVLVESHEKSLGEADKADVNVLTKAKSQ

SEQ ID NO: 2 - protein, 83 aa, Artificial Sequence
  Human PTH 1-83
SVSEIQLMHNLGKHLNSMERVEWLRKKLQDVHNFVALGAPLAPRDAGSQRPRKKEDNVLVESHEKSLGEADKADVNVLTKAKS

SEQ ID NO: 3 - protein, 82 aa, Artificial Sequence
  human PTH 1-82
SVSEIQLMHNLGKHLNSMERVEWLRKKLQDVHNFVALGAPLAPRDAGSQRPRKKEDNVLVESHEKSLGEADKADVNVLTKAK

SEQ ID NO: 4 - protein, 81 aa, Artificial Sequence
  human PTH 1-81
SVSEIQLMHNLGKHLNSMERVEWLRKKLQDVHNFVALGAPLAPRDAGSQRPRKKEDNVLVESHEKSLGEADKADVNVLTKA

SEQ ID NO: 5 - protein, 80 aa, Artificial Sequence
  human PTH 1-80
SVSEIQLMHNLGKHLNSMERVEWLRKKLQDVHNFVALGAPLAPRDAGSQRPRKKEDNVLVESHEKSLGEADKADVNVLTK

SEQ ID NO: 6 - protein, 79 aa, Artificial Sequence
  human PTH 1-79
SVSEIQLMHNLGKHLNSMERVEWLRKKLQDVHNFVALGAPLAPRDAGSQRPRKKEDNVLVESHEKSLGEADKADVNVLT

SEQ ID NO: 7 - protein, 78 aa, Artificial Sequence
  human PTH 1-78
SVSEIQLMHNLGKHLNSMERVEWLRKKLQDVHNFVALGAPLAPRDAGSQRPRKKEDNVLVESHEKSLGEADKADVNVL

SEQ ID NO: 8 - protein, 77 aa, Artificial Sequence
  human PTH 1-77
SVSEIQLMHNLGKHLNSMERVEWLRKKLQDVHNFVALGAPLAPRDAGSQRPRKKEDNVLVESHEKSLGEADKADVNV

SEQ ID NO: 9 - protein, 76 aa, Artificial Sequence
  human PTH 1-76
SVSEIQLMHNLGKHLNSMERVEWLRKKLQDVHNFVALGAPLAPRDAGSQRPRKKEDNVLVESHEKSLGEADKADVN

SEQ ID NO: 10 - protein, 75 aa, Artificial Sequence
  human PTH 1-75
SVSEIQLMHNLGKHLNSMERVEWLRKKLQDVHNFVALGAPLAPRDAGSQRPRKKEDNVLVESHEKSLGEADKADV

SEQ ID NO: 11 - protein, 74 aa, Artificial Sequence
  human PTH 1-74
SVSEIQLMHNLGKHLNSMERVEWLRKKLQDVHNFVALGAPLAPRDAGSQRPRKKEDNVLVESHEKSLGEADKAD

SEQ ID NO: 12 - protein, 73 aa, Artificial Sequence
  human PTH 1-73
SVSEIQLMHNLGKHLNSMERVEWLRKKLQDVHNFVALGAPLAPRDAGSQRPRKKEDNVLVESHEKSLGEADKA

SEQ ID NO: 13 - protein, 72 aa, Artificial Sequence
  human PTH 1-72
SVSEIQLMHNLGKHLNSMERVEWLRKKLQDVHNFVALGAPLAPRDAGSQRPRKKEDNVLVESHEKSLGEADK

SEQ ID NO: 14 - protein, 71 aa, Artificial Sequence
  human PTH 1-71
SVSEIQLMHNLGKHLNSMERVEWLRKKLQDVHNFVALGAPLAPRDAGSQRPRKKEDNVLVESHEKSLGEAD

SEQ ID NO: 15 - protein, 70 aa, Artificial Sequence
  human PTH 1-70
SVSEIQLMHNLGKHLNSMERVEWLRKKLQDVHNFVALGAPLAPRDAGSQRPRKKEDNVLVESHEKSLGEA

SEQ ID NO: 16 - protein, 69 aa, Artificial Sequence
  human PTH 1-69
SVSEIQLMHNLGKHLNSMERVEWLRKKLQDVHNFVALGAPLAPRDAGSQRPRKKEDNVLVESHEKSLGE

SEQ ID NO: 17 - protein, 68 aa, Artificial Sequence
  human PTH 1-68
SVSEIQLMHNLGKHLNSMERVEWLRKKLQDVHNFVALGAPLAPRDAGSQRPRKKEDNVLVESHEKSLG

SEQ ID NO: 18 - protein, 67 aa, Artificial Sequence
  human PTH 1-67
SVSEIQLMHNLGKHLNSMERVEWLRKKLQDVHNFVALGAPLAPRDAGSQRPRKKEDNVLVESHEKSL

SEQ ID NO: 19 - protein, 66 aa, Artificial Sequence
  human PTH 1-66
SVSEIQLMHNLGKHLNSMERVEWLRKKLQDVHNFVALGAPLAPRDAGSQRPRKKEDNVLVESHEKS

SEQ ID NO: 20 - protein, 65 aa, Artificial Sequence
  human PTH 1-65
SVSEIQLMHNLGKHLNSMERVEWLRKKLQDVHNFVALGAPLAPRDAGSQRPRKKEDNVLVESHEK

SEQ ID NO: 21 - protein, 64 aa, Artificial Sequence
  human PTH 1-64
SVSEIQLMHNLGKHLNSMERVEWLRKKLQDVHNFVALGAPLAPRDAGSQRPRKKEDNVLVESHE

SEQ ID NO: 22 - protein, 63 aa, Artificial Sequence
  human PTH 1-63
SVSEIQLMHNLGKHLNSMERVEWLRKKLQDVHNFVALGAPLAPRDAGSQRPRKKEDNVLVESH

SEQ ID NO: 23 - protein, 62 aa, Artificial Sequence
  human PTH 1-62
SVSEIQLMHNLGKHLNSMERVEWLRKKLQDVHNFVALGAPLAPRDAGSQRPRKKEDNVLVES

SEQ ID NO: 24 - protein, 61 aa, Artificial Sequence
  human PTH 1-61
SVSEIQLMHNLGKHLNSMERVEWLRKKLQDVHNFVALGAPLAPRDAGSQRPRKKEDNVLVE

SEQ ID NO: 25 - protein, 60 aa, Artificial Sequence
  human PTH 1-60
SVSEIQLMHNLGKHLNSMERVEWLRKKLQDVHNFVALGAPLAPRDAGSQRPRKKEDNVLV

SEQ ID NO: 26 - protein, 59 aa, Artificial Sequence
  human PTH 1-59
SVSEIQLMHNLGKHLNSMERVEWLRKKLQDVHNFVALGAPLAPRDAGSQRPRKKEDNVL

SEQ ID NO: 27 - protein, 58 aa, Artificial Sequence
  human PTH 1-58
SVSEIQLMHNLGKHLNSMERVEWLRKKLQDVHNFVALGAPLAPRDAGSQRPRKKEDNV

SEQ ID NO: 28 - protein, 57 aa, Artificial Sequence
  human PTH 1-57
SVSEIQLMHNLGKHLNSMERVEWLRKKLQDVHNFVALGAPLAPRDAGSQRPRKKEDN

SEQ ID NO: 29 - protein, 56 aa, Artificial Sequence
  human PTH 1-56
SVSEIQLMHNLGKHLNSMERVEWLRKKLQDVHNFVALGAPLAPRDAGSQRPRKKED

SEQ ID NO: 30 - protein, 55 aa, Artificial Sequence
  human PTH 1-55
SVSEIQLMHNLGKHLNSMERVEWLRKKLQDVHNFVALGAPLAPRDAGSQRPRKKE

SEQ ID NO: 31 - protein, 54 aa, Artificial Sequence
  human PTH 1-54
SVSEIQLMHNLGKHLNSMERVEWLRKKLQDVHNFVALGAPLAPRDAGSQRPRKK

SEQ ID NO: 32 - protein, 53 aa, Artificial Sequence
  human PTH 1-53
SVSEIQLMHNLGKHLNSMERVEWLRKKLQDVHNFVALGAPLAPRDAGSQRPRK

SEQ ID NO: 33 - protein, 52 aa, Artificial Sequence
  human PTH 1-52
SVSEIQLMHNLGKHLNSMERVEWLRKKLQDVHNFVALGAPLAPRDAGSQRPR

SEQ ID NO: 34 - protein, 51 aa, Artificial Sequence
  human PTH 1-51
SVSEIQLMHNLGKHLNSMERVEWLRKKLQDVHNFVALGAPLAPRDAGSQRP

SEQ ID NO: 35 - protein, 50 aa, Artificial Sequence
  human PTH 1-50
SVSEIQLMHNLGKHLNSMERVEWLRKKLQDVHNFVALGAPLAPRDAGSQR

SEQ ID NO: 36 - protein, 49 aa, Artificial Sequence
  human PTH 1-49
SVSEIQLMHNLGKHLNSMERVEWLRKKLQDVHNFVALGAPLAPRDAGSQ

SEQ ID NO: 37 - protein, 48 aa, Artificial Sequence
  human PTH 1-48
SVSEIQLMHNLGKHLNSMERVEWLRKKLQDVHNFVALGAPLAPRDAGS

SEQ ID NO: 38 - protein, 47 aa, Artificial Sequence
  human PTH 1-47
SVSEIQLMHNLGKHLNSMERVEWLRKKLQDVHNFVALGAPLAPRDAG

SEQ ID NO: 39 - protein, 46 aa, Artificial Sequence
  human PTH 1-46
SVSEIQLMHNLGKHLNSMERVEWLRKKLQDVHNFVALGAPLAPRDA

SEQ ID NO: 40 - protein, 45 aa, Artificial Sequence
  human PTH 1-45
SVSEIQLMHNLGKHLNSMERVEWLRKKLQDVHNFVALGAPLAPRD

SEQ ID NO: 41 - protein, 44 aa, Artificial Sequence
  human PTH 1-44
SVSEIQLMHNLGKHLNSMERVEWLRKKLQDVHNFVALGAPLAPR

SEQ ID NO: 42 - protein, 43 aa, Artificial Sequence
  human PTH 1-43
SVSEIQLMHNLGKHLNSMERVEWLRKKLQDVHNFVALGAPLAP

SEQ ID NO: 43 - protein, 42 aa, Artificial Sequence
  human PTH 1-42
SVSEIQLMHNLGKHLNSMERVEWLRKKLQDVHNFVALGAPLA

SEQ ID NO: 44 - protein, 41 aa, Artificial Sequence
  human PTH-41
SVSEIQLMHNLGKHLNSMERVEWLRKKLQDVHNFVALGAPL

SEQ ID NO: 45 - protein, 40 aa, Artificial Sequence
  human PTH 1-40
SVSEIQLMHNLGKHLNSMERVEWLRKKLQDVHNFVALGAP

SEQ ID NO: 46 - protein, 39 aa, Artificial Sequence
  human PTH 1-39
SVSEIQLMHNLGKHLNSMERVEWLRKKLQDVHNFVALGA

SEQ ID NO: 47 - protein, 38 aa, Artificial Sequence
  human PTH 1-38
SVSEIQLMHNLGKHLNSMERVEWLRKKLQDVHNFVALG

SEQ ID NO: 48 - protein, 37 aa, Artificial Sequence
  human PTH 1-37
SVSEIQLMHNLGKHLNSMERVEWLRKKLQDVHNFVAL

SEQ ID NO: 49 - protein, 36 aa, Artificial Sequence
  human PTH 1-36
SVSEIQLMHNLGKHLNSMERVEWLRKKLQDVHNFVA

SEQ ID NO: 50 - protein, 35 aa, Artificial Sequence
  human PTH 1-35
SVSEIQLMHNLGKHLNSMERVEWLRKKLQDVHNFV

SEQ ID NO: 51 - protein, 34 aa, Artificial Sequence
  human PTH 1-34
SVSEIQLMHNLGKHLNSMERVEWLRKKLQDVHNF

SEQ ID NO: 52 - protein, 33 aa, Artificial Sequence
  human PTH 1-33
SVSEIQLMHNLGKHLNSMERVEWLRKKLQDVHN

SEQ ID NO: 53 - protein, 32 aa, Artificial Sequence
  human PTH 1-32
SVSEIQLMHNLGKHLNSMERVEWLRKKLQDVH

SEQ ID NO: 54 - protein, 31 aa, Artificial Sequence
  human PTH 1-31
SVSEIQLMHNLGKHLNSMERVEWLRKKLQDV

SEQ ID NO: 55 - protein, 30 aa, Artificial Sequence
  human PTH 1-30
SVSEIQLMHNLGKHLNSMERVEWLRKKLQD

SEQ ID NO: 56 - protein, 29 aa, Artificial Sequence
  human PTH 1-29
SVSEIQLMHNLGKHLNSMERVEWLRKKLQ

SEQ ID NO: 57 - protein, 28 aa, Artificial Sequence
  human PTH 1-28
SVSEIQLMHNLGKHLNSMERVEWLRKKL

SEQ ID NO: 58 - protein, 27 aa, Artificial Sequence
  human PTH 1-27
SVSEIQLMHNLGKHLNSMERVEWLRKK

SEQ ID NO: 59 - protein, 26 aa, Artificial Sequence
  human PTH 1-26
SVSEIQLMHNLGKHLNSMERVEWLRK

SEQ ID NO: 60 - protein, 25 aa, Artificial Sequence
  human PTH 1-25
SVSEIQLMHNLGKHLNSMERVEWLR

SEQ ID NO: 61 - protein, 84 aa, Artificial Sequence; identical to SEQ ID NO: 1
  amidated human PTH 1-84
  MOD_RES (84)..(84): AMIDATION

SEQ ID NO: 62 - protein, 83 aa, Artificial Sequence; identical to SEQ ID NO: 2
  amidated human PTH 1-83
  MOD_RES (83)..(83): AMIDATION

SEQ ID NO: 63 - protein, 82 aa, Artificial Sequence; identical to SEQ ID NO: 3
  amidated human PTH 1-82
  MOD_RES (82)..(82): AMIDATION

SEQ ID NO: 64 - protein, 81 aa, Artificial Sequence; identical to SEQ ID NO: 4
  amidated human PTH 1-81
  MOD_RES (81)..(81): AMIDATION

SEQ ID NO: 65 - protein, 80 aa, Artificial Sequence; identical to SEQ ID NO: 5
  amidated human PTH 1-80
  MOD_RES (80)..(80): AMIDATION

SEQ ID NO: 66 - protein, 79 aa, Artificial Sequence; identical to SEQ ID NO: 6
  amidated human PTH 1-79
  MOD_RES (79)..(79): AMIDATION

SEQ ID NO: 67 - protein, 78 aa, Artificial Sequence; identical to SEQ ID NO: 7
  amidated human PTH 1-78
  MOD_RES (78)..(78): AMIDATION

SEQ ID NO: 68 - protein, 77 aa, Artificial Sequence; identical to SEQ ID NO: 8
  amidated human PTH 1-77
  MOD_RES (77)..(77): AMIDATION

SEQ ID NO: 69 - protein, 76 aa, Artificial Sequence; identical to SEQ ID NO: 9
  amidated human PTH 1-76
  MOD_RES (76)..(76): AMIDATION

SEQ ID NO: 70 - protein, 75 aa, Artificial Sequence; identical to SEQ ID NO: 10
  amidated human PTH 1-75
  MOD_RES (75)..(75): AMIDATION

SEQ ID NO: 71 - protein, 74 aa, Artificial Sequence; identical to SEQ ID NO: 11
  amidated human PTH 1-74
  MOD_RES (74)..(74): AMIDATION

SEQ ID NO: 72 - protein, 73 aa, Artificial Sequence; identical to SEQ ID NO: 12
  amidated human PTH 1-73
  MOD_RES (73)..(73): AMIDATION

SEQ ID NO: 73 - protein, 72 aa, Artificial Sequence; identical to SEQ ID NO: 13
  amidated human PTH 1-72
  MOD_RES (72)..(72): AMIDATION

SEQ ID NO: 74 - protein, 71 aa, Artificial Sequence; identical to SEQ ID NO: 14
  amidated human PTH 1-71
  MOD_RES (71)..(71): AMIDATION

SEQ ID NO: 75 - protein, 70 aa, Artificial Sequence; identical to SEQ ID NO: 15
  amidated human PTH 1-70
  MOD_RES (70)..(70): AMIDATION

SEQ ID NO: 76 - protein, 69 aa, Artificial Sequence; identical to SEQ ID NO: 16
  amidated human PTH 1-69
  MOD_RES (69)..(69): AMIDATION

SEQ ID NO: 77 - protein, 68 aa, Artificial Sequence; identical to SEQ ID NO: 17
  amidated human PTH 1-68
  MOD_RES (68)..(68): AMIDATION

SEQ ID NO: 78 - protein, 67 aa, Artificial Sequence; identical to SEQ ID NO: 18
  amidated human PTH 1-67
  MOD_RES (67)..(67): AMIDATION

SEQ ID NO: 79 - protein, 66 aa, Artificial Sequence; identical to SEQ ID NO: 19
  amidated human PTH 1-66
  MOD_RES (66)..(66): AMIDATION

SEQ ID NO: 80 - protein, 65 aa, Artificial Sequence; identical to SEQ ID NO: 20
  amidated human PTH 1-65
  MOD_RES (65)..(65): AMIDATION

SEQ ID NO: 81 - protein, 64 aa, Artificial Sequence; identical to SEQ ID NO: 21
  amidated human PTH 1-64
  MOD_RES (64)..(64): AMIDATION

SEQ ID NO: 82 - protein, 63 aa, Artificial Sequence; identical to SEQ ID NO: 22
  amidated human PTH 1-63
  MOD_RES (63)..(63): AMIDATION

SEQ ID NO: 83 - protein, 62 aa, Artificial Sequence; identical to SEQ ID NO: 23
  amidated human PTH 1-62
  MOD_RES (62)..(62): AMIDATION

SEQ ID NO: 84 - protein, 61 aa, Artificial Sequence; identical to SEQ ID NO: 24
  amidated human PTH 1-61
  MOD_RES (61)..(61): AMIDATION

SEQ ID NO: 85 - protein, 60 aa, Artificial Sequence; identical to SEQ ID NO: 25
  amidated human PTH 1-60
  MOD_RES (60)..(60): ACETYLATION

SEQ ID NO: 86 - protein, 59 aa, Artificial Sequence; identical to SEQ ID NO: 26
  amidated human PTH 1-59
  MOD_RES (59)..(59): AMIDATION

SEQ ID NO: 87 - protein, 58 aa, Artificial Sequence; identical to SEQ ID NO: 27
  amidated human PTH 1-58
  MOD_RES (58)..(58): AMIDATION

SEQ ID NO: 88 - protein, 57 aa, Artificial Sequence; identical to SEQ ID NO: 28
  amidated human PTH 1-57
  MOD_RES (57)..(57): AMIDATION

SEQ ID NO: 89 - protein, 56 aa, Artificial Sequence; identical to SEQ ID NO: 29
  amidated human PTH 1-56
  MOD_RES (56)..(56): AMIDATION

SEQ ID NO: 90 - protein, 55 aa, Artificial Sequence; identical to SEQ ID NO: 30
  amidated human PTH 1-55
  MOD_RES (55)..(55): AMIDATION

SEQ ID NO: 91 - protein, 54 aa, Artificial Sequence; identical to SEQ ID NO: 31
  amidated human PTH 1-54
  MOD_RES (54)..(54): AMIDATION

SEQ ID NO: 92 - protein, 53 aa, Artificial Sequence; identical to SEQ ID NO: 32
  amidated human PTH 1-53
  MOD_RES (53)..(53): AMIDATION

SEQ ID NO: 93 - protein, 52 aa, Artificial Sequence; identical to SEQ ID NO: 33
  amidated human PTH 1-52
  MOD_RES (52)..(52): AMIDATION

SEQ ID NO: 94 - protein, 51 aa, Artificial Sequence; identical to SEQ ID NO: 34
  amidated human PTH 1-51
  MOD_RES (51)..(51): AMIDATION

SEQ ID NO: 95 - protein, 50 aa, Artificial Sequence; identical to SEQ ID NO: 35
  amidated human PTH 1-50
  MOD_RES (50)..(50): AMIDATION

SEQ ID NO: 96 - protein, 49 aa, Artificial Sequence; identical to SEQ ID NO: 36
  amidated human PTH 1-49
  MOD_RES (49)..(49): AMIDATION

SEQ ID NO: 97 - protein, 48 aa, Artificial Sequence; identical to SEQ ID NO: 37
  amidated human PTH 1-48
  MOD_RES (48)..(48): AMIDATION

SEQ ID NO: 98 - protein, 47 aa, Artificial Sequence; identical to SEQ ID NO: 38
  amidated human PTH 1-47
  MOD_RES (47)..(47): AMIDATION

SEQ ID NO: 99 - protein, 46 aa, Artificial Sequence; identical to SEQ ID NO: 39
  amidated human PTH 1-46
  MOD_RES (46)..(46): AMIDATION

SEQ ID NO: 100 - protein, 45 aa, Artificial Sequence; identical to SEQ ID NO: 40
  amidated human PTH 1-45
  MOD_RES (45)..(45): AMIDATION

SEQ ID NO: 101 - protein, 44 aa, Artificial Sequence; identical to SEQ ID NO: 41
  amidated human PTH 1-44
  MOD_RES (44)..(44): AMIDATION

SEQ ID NO: 102 - protein, 43 aa, Artificial Sequence; identical to SEQ ID NO: 42
  amidated human PTH 1-43
  MOD_RES (43)..(43): AMIDATION

SEQ ID NO: 103 - protein, 42 aa, Artificial Sequence; identical to SEQ ID NO: 43
  amidated human PTH 1-42
  MOD_RES (42)..(42): AMIDATION

SEQ ID NO: 104 - protein, 41 aa, Artificial Sequence; identical to SEQ ID NO: 44
  amidated human PTH 1-41
  MOD_RES (41)..(41): AMIDATION

SEQ ID NO: 105 - protein, 40 aa, Artificial Sequence; identical to SEQ ID NO: 45
  amidated human PTH 1-40
  MOD_RES (40)..(40): AMIDATION

SEQ ID NO: 106 - protein, 39 aa, Artificial Sequence; identical to SEQ ID NO: 46
  amidated human PTH 1-39
  MOD_RES (39)..(39): AMIDATION

SEQ ID NO: 107 - protein, 38 aa, Artificial Sequence; identical to SEQ ID NO: 47
  amidated human PTH 1-38
  MOD_RES (38)..(38): AMIDATION

SEQ ID NO: 108 - protein, 37 aa, Artificial Sequence; identical to SEQ ID NO: 48
  amidated human PTH 1-37
  MOD_RES (37)..(37): AMIDATION

SEQ ID NO: 109 - protein, 36 aa, Artificial Sequence; identical to SEQ ID NO: 49
  amidated human PTH 1-36
  MOD_RES (36)..(36): AMIDATION

SEQ ID NO: 110 - protein, 35 aa, Artificial Sequence; identical to SEQ ID NO: 50
  amidated human PTH 1-35
  MOD_RES (35)..(35): AMIDATION

SEQ ID NO: 111 - protein, 34 aa, Artificial Sequence; identical to SEQ ID NO: 51
  amidated human PTH 1-34
  MOD_RES (34)..(34): AMIDATION

SEQ ID NO: 112 - protein, 33 aa, Artificial Sequence; identical to SEQ ID NO: 52
  amidated human PTH 1-33
  MOD_RES (33)..(33): AMIDATION

SEQ ID NO: 113 - protein, 32 aa, Artificial Sequence; identical to SEQ ID NO: 53
  amidated human PTH 1-32
  MOD_RES (32)..(32): AMIDATION

SEQ ID NO: 114 - protein, 31 aa, Artificial Sequence; identical to SEQ ID NO: 54
  amidated human PTH 1-31
  MOD_RES (31)..(31): AMIDATION

SEQ ID NO: 115 - protein, 30 aa, Artificial Sequence; identical to SEQ ID NO: 55
  amidated human PTH 1-30
  MOD_RES (30)..(30): AMIDATION

SEQ ID NO: 116 - protein, 29 aa, Artificial Sequence
  amidated human PTH 1-29
  MOD_RES (29)..(29): AMIDATION
SVSEIQLMHNLGKHLNSMERVEWLRKKLQ

SEQ ID NO: 117 - protein, 28 aa, Artificial Sequence
  amidated human PTH 1-28
  MOD_RES (28)..(28): AMIDATION
SVSEIQLMHNLGKHLNSMERVEWLRKKL

SEQ ID NO: 118 - protein, 27 aa, Artificial Sequence
  amidated human PTH 1-27
  MOD_RES (27)..(27): AMIDATION
SVSEIQLMHNLGKHLNSMERVEWLRKK

SEQ ID NO: 119 - protein, 26 aa, Artificial Sequence
  amidated human PTH 1-26
  MOD_RES (26)..(26): AMIDATION
SVSEIQLMHNLGKHLNSMERVEWLRK

SEQ ID NO: 120 - protein, 25 aa, Artificial Sequence
  amidated human PTH 1-25
  MOD_RES (25)..(25): AMIDATION
SVSEIQLMHNLGKHLNSMERVEWLR

SEQ ID NO: 121 - protein, 141 aa, Homo sapiens
AVSEHQLLHDKGKSIQDLRRRFFLHHLIAEIHTAEIRATSEVSPNSKPSPNTKNHPVRFGSDDEGRYLTQETNKVETYKEQPLKTPGKKKKGKPGKRKEQEKKKRRTRSAWLDSGVTGSGLEGDHLSDTSTTSLELDSRRH

SEQ ID NO: 122 - protein, 20 aa, Artificial Sequence
  Artificial random coil
GGPGGPGPGGPGGPGPGGPG